European Patent Application EP 4 410 274 A1, published August 7, 2024. Title: PHARMACEUTICAL COMPOSITION FOR TREATING INFLAMMATORY DISEASE. Applicant: INDUSTRY FOUNDATION OF CHONNAM NATIONAL UNIVERSITY. The sequence listing filed with the application follows.

SEQUENCE LISTING (14 sequences)

SEQ ID NO: 1 - DNA, 24 bp, Artificial Sequence
  Ccl2(MCP-1) forward
atcccaatgagtaggctggagagc

SEQ ID NO: 2 - DNA, 23 bp, Artificial Sequence
  Ccl2(MCP-1) reverse
cagaagtgcttgaggtggttgtg

SEQ ID NO: 3 - DNA, 20 bp, Artificial Sequence
  Gapdh forward
tgtgtccgtcgtggatctga

SEQ ID NO: 4 - DNA, 20 bp, Artificial Sequence
  Gapdh reverse
gatgcctgcttcaccacctt

SEQ ID NO: 5 - DNA, 21 bp, Artificial Sequence
  Icam1 forward
aacttttcagctccggtcctg

SEQ ID NO: 6 - DNA, 21 bp, Artificial Sequence
  Icam1 reverse
tcagtgtgaattggacctgcg

SEQ ID NO: 7 - DNA, 22 bp, Artificial Sequence
  Il-6 forward
acaaccacggccttccctactt

SEQ ID NO: 8 - DNA, 23 bp, Artificial Sequence
  Il-6 reverse
cacgatttcccagagaacatgtg

SEQ ID NO: 9 - DNA, 24 bp, Artificial Sequence
  Tgfb1(TGFbeta) forward
caacaattcctggcgttaccttgg

SEQ ID NO: 10 - DNA, 24 bp, Artificial Sequence
  Tgfb1(TGFbeta) reverse
gaaagccctgtattccgtctcctt

SEQ ID NO: 11 - DNA, 20 bp, Artificial Sequence
  Tnf(TNFalpha) forward
gcatgatccgcgacgtggaa

SEQ ID NO: 12 - DNA, 20 bp, Artificial Sequence
  Tnf(TNFalpha) reverse
agatccatgccgttggccag

SEQ ID NO: 13 - DNA, 20 bp, Artificial Sequence
  Vcam1 forward
tctctcaggaaatgccaccc

SEQ ID NO: 14 - DNA, 20 bp, Artificial Sequence
  Vcam1 reverse
cacagccaatagcagcacac